European Patent Specification EP 3 309 176 B1, published October 1, 2025. Title: AMINO ACID SEQUENCES DIRECTED AGAINST OX40L AND POLYPEPTIDES COMPRISING THE SAME FOR THE TREATMENT OF ASTHMA. Applicant: Ablynx N.V. Ablynx N.V. The sequence listing filed with the application follows.

SEQUENCE LISTING (234 sequences)

SEQ ID NO: 1 - protein, 102 aa, Artificial Sequence
  KERE-class Nanobody
  misc_feature (31)..(35): CDR
  misc_feature (50)..(54): CDR
  misc_feature (87)..(91): CDR
EVQLVESGGGLVQPGGSLRLSCAASGIPFSXXXXXWFRQAPGKQRDSVAXXXXXRFTISRDNAKNTVYLQMNSLKPEDTAVYRCYFXXXXXWGQGTQVTVSS

SEQ ID NO: 2 - protein, 102 aa, Artificial Sequence
  KERE-class Nanobody
  misc_feature (31)..(35): CDR
  misc_feature (50)..(54): CDR
  misc_feature (87)..(91): CDR
QVKLEESGGGLVQAGGSLRLSCVGSGRTFSXXXXXWFRLAPGKEREFVAXXXXXRFTISRDTASNRGYLHMNNLTPEDTAVYYCAAXXXXXWGQGTQVTVSS

SEQ ID NO: 3 - protein, 102 aa, Artificial Sequence
  KERE-class Nanobody
  misc_feature (31)..(35): CDR
  misc_feature (50)..(54): CDR
  misc_feature (87)..(91): CDR
AVQLVDSGGGLVQAGDSLKLSCALTGGAFTXXXXXWFRQTPGREREFVAXXXXXRFTISRDNAKNMVYLRMNSLIPEDAAVYSCAAXXXXXWGQGTLVTVSS

SEQ ID NO: 4 - protein, 102 aa, Artificial Sequence
  KERE-class Nanobody
  misc_feature (31)..(35): CDR
  misc_feature (50)..(54): CDR
  misc_feature (87)..(91): CDR
QVQLVESGGGLVEAGGSLRLSCTASESPFRXXXXXWFRQTSGQEREFVAXXXXXRFTISRDDAKNTVWLHGSTLKPEDTAVYYCAAXXXXXWGQGTQVTVSS

SEQ ID NO: 5 - protein, 102 aa, Artificial Sequence
  KERE-class Nanobody
  misc_feature (31)..(35): CDR
  misc_feature (50)..(54): CDR
  misc_feature (87)..(91): CDR
AVQLVESGGGLVQGGGSLRLACAASERIFDXXXXXWYRQGPGNERELVAXXXXXRFTISMDYTKQTVYLHMNSLRPEDTGLYYCKIXXXXXWGQGTQVTVSS

SEQ ID NO: 6 - protein, 102 aa, Artificial Sequence
  KERE-class Nanobody
  misc_feature (31)..(35): CDR
  misc_feature (50)..(54): CDR
  misc_feature (87)..(91): CDR
DVKFVESGGGLVQAGGSLRLSCVASGFNFDXXXXXWFRQAPGKEREEVAXXXXXRFTISSEKDKNSVYLQMNSLKPEDTALYICAGXXXXXWGRGTQVTVSS

SEQ ID NO: 7 - protein, 102 aa, Artificial Sequence
  KERE-class Nanobody
  misc_feature (31)..(35): CDR
  misc_feature (50)..(54): CDR
  misc_feature (87)..(91): CDR
QVRLAESGGGLVQSGGSLRLSCVASGSTYTXXXXXWYRQYPGKQRALVAXXXXXRFTIARDSTKDTFCLQMNNLKPEDTAVYYCYAXXXXXWGQGTQVTVSS

SEQ ID NO: 8 - protein, 102 aa, Artificial Sequence
  KERE-class Nanobody
  misc_feature (31)..(35): CDR
  misc_feature (50)..(54): CDR
  misc_feature (87)..(91): CDR
EVQLVESGGGLVQAGGSLRLSCAASGFTSDXXXXXWFRQAPGKPREGVSXXXXXRFTISTDNAKNTVHLLMNRVNAEDTALYYCAVXXXXXWGRGTRVTVSS

SEQ ID NO: 9 - protein, 102 aa, Artificial Sequence
  KERE-class Nanobody
  misc_feature (31)..(35): CDR
  misc_feature (50)..(54): CDR
  misc_feature (87)..(91): CDR
QVQLVESGGGLVQPGGSLRLSCQASGDISTXXXXXWYRQVPGKLREFVAXXXXXRFTISGDNAKRAIYLQMNNLKPDDTAVYYCNRXXXXXWGQGTQVTVSP

SEQ ID NO: 10 - protein, 102 aa, Artificial Sequence
  KERE-class Nanobody
  misc_feature (31)..(35): CDR
  misc_feature (50)..(54): CDR
  misc_feature (87)..(91): CDR
QVPVVESGGGLVQAGDSLRLFCAVPSFTSTXXXXXWFRQAPGKEREFVAXXXXXRFTISRNATKNTLTLRMDSLKPEDTAVYYCAAXXXXXWGQGTQVTVSS

SEQ ID NO: 11 - protein, 102 aa, Artificial Sequence
  KERE-class Nanobody
  misc_feature (31)..(35): CDR
  misc_feature (50)..(54): CDR
  misc_feature (87)..(91): CDR
EVQLVESGGGLVQAGDSLRLFCTVSGGTASXXXXXWFRQAPGEKREFVAXXXXXRFTIARENAGNMVYLQMNNLKPDDTALYTCAAXXXXXWGRGTQVTVSS

SEQ ID NO: 12 - protein, 102 aa, Artificial Sequence
  KERE-class Nanobody
  misc_feature (31)..(35): CDR
  misc_feature (50)..(54): CDR
  misc_feature (87)..(91): CDR
AVQLVESGGDSVQPGDSQTLSCAASGRTNSXXXXXWFRQAPGKERVFLAXXXXXRFTISRDSAKNMMYLQMNNLKPQDTAVYYCAAXXXXXWGQGTQVTVSS

SEQ ID NO: 13 - protein, 102 aa, Artificial Sequence
  KERE-class Nanobody
  misc_feature (31)..(35): CDR
  misc_feature (50)..(54): CDR
  misc_feature (87)..(91): CDR
AVQLVESGGGLVQAGGSLRLSCVVSGLTSSXXXXXWFRQTPWQERDFVAXXXXXRFTISRDNYKDTVLLEMNFLKPEDTAIYYCAAXXXXXWGQGTQVTVSS

SEQ ID NO: 14 - protein, 102 aa, Artificial Sequence
  KERE-class Nanobody
  misc_feature (31)..(35): CDR
  misc_feature (50)..(54): CDR
  misc_feature (87)..(91): CDR
AVQLVESGGGLVQAGASLRLSCATSTRTLDXXXXXWFRQAPGRDREFVAXXXXXRFTVSRDSAENTVALQMNSLKPEDTAVYYCAAXXXXXWGQGTRVTVSS

SEQ ID NO: 15 - protein, 102 aa, Artificial Sequence
  KERE-class Nanobody
  misc_feature (31)..(35): CDR
  misc_feature (50)..(54): CDR
  misc_feature (87)..(91): CDR
QVQLVESGGGLVQPGGSLRLSCTVSRLTAHXXXXXWFRQAPGKEREAVSXXXXXRFTISRDYAGNTAFLQMDSLKPEDTGVYYCATXXXXXWGQGTQVTVSS

SEQ ID NO: 16 - protein, 102 aa, Artificial Sequence
  KERE-class Nanobody
  misc_feature (31)..(35): CDR
  misc_feature (50)..(54): CDR
  misc_feature (87)..(91): CDR
EVQLVESGGELVQAGGSLKLSCTASGRNFVXXXXXWFRRAPGKEREFVAXXXXXRFTVSRDNGKNTAYLRMNSLKPEDTADYYCAVXXXXXLGSGTQVTVSS

SEQ ID NO: 17 - protein, 102 aa, Artificial Sequence
  GLEW-class Nanobody
  misc_feature (31)..(35): CDR
  misc_feature (50)..(54): CDR
  misc_feature (87)..(91): CDR
AVQLVESGGGLVQPGGSLRLSCAASGFTFSXXXXXWVRQAPGKVLEWVSXXXXXRFTISRDNAKNTLYLQMNSLKPEDTAVYYCVKXXXXXGSQGTQVTVSS

SEQ ID NO: 18 - protein, 102 aa, Artificial Sequence
  GLEW-class Nanobody
  misc_feature (31)..(35): CDR
  misc_feature (50)..(54): CDR
  misc_feature (87)..(91): CDR
EVQLVESGGGLVQPGGSLRLSCVCVSSGCTXXXXXWVRQAPGKAEEWVSXXXXXRFKISRDNAKKTLYLQMNSLGPEDTAMYYCQRXXXXXRGQGTQVTVSS

SEQ ID NO: 19 - protein, 102 aa, Artificial Sequence
  GLEW-class Nanobody
  misc_feature (31)..(35): CDR
  misc_feature (50)..(54): CDR
  misc_feature (87)..(91): CDR
EVQLVESGGGLALPGGSLTLSCVFSGSTFSXXXXXWVRHTPGKAEEWVSXXXXXRFTISRDNAKNTLYLEMNSLSPEDTAMYYCGRXXXXXRSKGIQVTVSS

SEQ ID NO: 20 - protein, 102 aa, Artificial Sequence
  P,R,S 103-class Nanobody
  misc_feature (31)..(35): CDR
  misc_feature (50)..(54): CDR
  misc_feature (87)..(91): CDR
AVQLVESGGGLVQAGGSLRLSCAASGRTFSXXXXXWFRQAPGKEREFVAXXXXXRFTISRDNAKNTVYLQMNSLKPEDTAVYYCAAXXXXXRGQGTQVTVSS

SEQ ID NO: 21 - protein, 102 aa, Artificial Sequence
  P,R,S 103-class Nanobody
  misc_feature (31)..(35): CDR
  misc_feature (50)..(54): CDR
  misc_feature (87)..(91): CDR
DVQLVESGGDLVQPGGSLRLSCAASGFSFDXXXXXWLRQTPGKGLEWVGXXXXXRFTISRDNAKNMLYLHLNNLKSEDTAVYYCRRXXXXXLGQGTQVTVSS

SEQ ID NO: 22 - protein, 102 aa, Artificial Sequence; identical to SEQ ID NO: 18
  P,R,S 103-class Nanobody
  misc_feature (31)..(35): CDR
  misc_feature (50)..(54): CDR
  misc_feature (87)..(91): CDR

SEQ ID NO: 23 - protein, 30 aa, Artificial Sequence
  KERE-class Nanobody FW1 sequence
QVQRVESGGGLVQAGGSLRLSCAASGRTSS

SEQ ID NO: 24 - protein, 30 aa, Artificial Sequence
  KERE-class Nanobody FW1 sequence
QVQLVESGGGLVQTGDSLSLSCSASGRTFS

SEQ ID NO: 25 - protein, 30 aa, Artificial Sequence
  KERE-class Nanobody FW1 sequence
QVKLEESGGGLVQAGDSLRLSCAATGRAFG

SEQ ID NO: 26 - protein, 30 aa, Artificial Sequence
  KERE-class Nanobody FW1 sequence
AVQLVESGGGLVQPGESLGLSCVASGRDFV

SEQ ID NO: 27 - protein, 30 aa, Artificial Sequence
  KERE-class Nanobody FW1 sequence
EVQLVESGGGLVQAGGSLRLSCEVLGRTAG

SEQ ID NO: 28 - protein, 30 aa, Artificial Sequence
  KERE-class Nanobody FW1 sequence
QVQLVESGGGWVQPGGSLRLSCAASETILS

SEQ ID NO: 29 - protein, 30 aa, Artificial Sequence
  KERE-class Nanobody FW1 sequence
QVQLVESGGGTVQPGGSLNLSCVASGNTFN

SEQ ID NO: 30 - protein, 30 aa, Artificial Sequence
  KERE-class Nanobody FW1 sequence
EVQLVESGGGLAQPGGSLQLSCSAPGFTLD

SEQ ID NO: 31 - protein, 30 aa, Artificial Sequence
  KERE-class Nanobody FW1 sequence
AQELEESGGGLVQAGGSLRLSCAASGRTFN

SEQ ID NO: 32 - protein, 22 aa, Artificial Sequence
  KERE-class Nanobody FW1 sequence
VESGGGLVQPGGSLRLSCAASG

SEQ ID NO: 33 - protein, 22 aa, Artificial Sequence
  KERE-class Nanobody FW1 sequence
VDSGGGLVQAGDSLKLSCALTG

SEQ ID NO: 34 - protein, 22 aa, Artificial Sequence
  KERE-class Nanobody FW1 sequence
VDSGGGLVQAGDSLRLSCAASG

SEQ ID NO: 35 - protein, 22 aa, Artificial Sequence
  KERE-class Nanobody FW1 sequence
VDSGGGLVEAGGSLRLSCQVSE

SEQ ID NO: 36 - protein, 22 aa, Artificial Sequence
  KERE-class Nanobody FW1 sequence
QDSGGGSVQAGGSLKLSCAASG

SEQ ID NO: 37 - protein, 22 aa, Artificial Sequence
  KERE-class Nanobody FW1 sequence
VQSGGRLVQAGDSLRLSCAASE

SEQ ID NO: 38 - protein, 22 aa, Artificial Sequence
  KERE-class Nanobody FW1 sequence
VESGGTLVQSGDSLKLSCASST

SEQ ID NO: 39 - protein, 22 aa, Artificial Sequence
  KERE-class Nanobody FW1 sequence
MESGGDSVQSGGSLTLSCVASG

SEQ ID NO: 40 - protein, 22 aa, Artificial Sequence
  KERE-class Nanobody FW1 sequence
QASGGGLVQAGGSLRLSCSASV

SEQ ID NO: 41 - protein, 14 aa, Artificial Sequence
  KERE-class Nanobody FW2 sequence
WFRQAPGKEREFVA

SEQ ID NO: 42 - protein, 14 aa, Artificial Sequence
  KERE-class Nanobody FW2 sequence
WFRQTPGREREFVA

SEQ ID NO: 43 - protein, 14 aa, Artificial Sequence
  KERE-class Nanobody FW2 sequence
WYRQAPGKQREMVA

SEQ ID NO: 44 - protein, 14 aa, Artificial Sequence
  KERE-class Nanobody FW2 sequence
WYRQGPGKQRELVA

SEQ ID NO: 45 - protein, 14 aa, Artificial Sequence
  KERE-class Nanobody FW2 sequence
WIRQAPGKEREGVS

SEQ ID NO: 46 - protein, 14 aa, Artificial Sequence
  KERE-class Nanobody FW2 sequence
WFREAPGKEREGIS

SEQ ID NO: 47 - protein, 14 aa, Artificial Sequence
  KERE-class Nanobody FW2 sequence
WYRQAPGKERDLVA

SEQ ID NO: 48 - protein, 14 aa, Artificial Sequence
  KERE-class Nanobody FW2 sequence
WFRQAPGKQREEVS

SEQ ID NO: 49 - protein, 14 aa, Artificial Sequence
  KERE-class Nanobody FW2 sequence
WFRQPPGKVREFVG

SEQ ID NO: 50 - protein, 32 aa, Artificial Sequence
  KERE-class Nanobody FW3 sequence
RFTISRDNAKNTVYLQMNSLKPEDTAVYRCYF

SEQ ID NO: 51 - protein, 32 aa, Artificial Sequence
  KERE-class Nanobody FW3 sequence
RFAISRDNNKNTGYLQMNSLEPEDTAVYYCAA

SEQ ID NO: 52 - protein, 32 aa, Artificial Sequence
  KERE-class Nanobody FW3 sequence
RFTVARNNAKNTVNLEMNSLKPEDTAVYYCAA

SEQ ID NO: 53 - protein, 32 aa, Artificial Sequence
  KERE-class Nanobody FW3 sequence
RFTISRDIAKNTVDLLMNNLEPEDTAVYYCAA

SEQ ID NO: 54 - protein, 32 aa, Artificial Sequence
  KERE-class Nanobody FW3 sequence
RLTISRDNAVDTMYLQMNSLKPEDTAVYYCAA

SEQ ID NO: 55 - protein, 32 aa, Artificial Sequence
  KERE-class Nanobody FW3 sequence
RFTISRDNAKNTVYLQMDNVKPEDTAIYYCAA

SEQ ID NO: 56 - protein, 32 aa, Artificial Sequence
  KERE-class Nanobody FW3 sequence
RFTISKDSGKNTVYLQMTSLKPEDTAVYYCAT

SEQ ID NO: 57 - protein, 32 aa, Artificial Sequence
  KERE-class Nanobody FW3 sequence
RFTISRDSAKNMMYLQMNNLKPQDTAVYYCAA

SEQ ID NO: 58 - protein, 32 aa, Artificial Sequence
  KERE-class Nanobody FW3 sequence
RFTISRENDKSTVYLQLNSLKPEDTAVYYCAA

SEQ ID NO: 59 - protein, 32 aa, Artificial Sequence
  KERE-class Nanobody FW3 sequence
RFTISRDYAGNTAYLQMNSLKPEDTGVYYCAT

SEQ ID NO: 60 - protein, 11 aa, Artificial Sequence
  KERE-class Nanobody FW4 sequence
WGQGTQVTVSS

SEQ ID NO: 61 - protein, 11 aa, Artificial Sequence
  KERE-class Nanobody FW4 sequence
WGKGTLVTVSS

SEQ ID NO: 62 - protein, 11 aa, Artificial Sequence
  KERE-class Nanobody FW4 sequence
RGQGTRVTVSS

SEQ ID NO: 63 - protein, 11 aa, Artificial Sequence
  KERE-class Nanobody FW4 sequence
WGLGTQVTISS

SEQ ID NO: 64 - protein, 30 aa, Artificial Sequence
  GLEW-class Nanobody FW1 sequence
QVQLVESGGGLVQPGGSLRLSCAASGFTFS

SEQ ID NO: 65 - protein, 30 aa, Artificial Sequence
  GLEW-class Nanobody FW1 sequence
EVHLVESGGGLVRPGGSLRLSCAAFGFIFK

SEQ ID NO: 66 - protein, 30 aa, Artificial Sequence
  GLEW-class Nanobody FW1 sequence
QVKLEESGGGLAQPGGSLRLSCVASGFTFS

SEQ ID NO: 67 - protein, 30 aa, Artificial Sequence
  GLEW-class Nanobody FW1 sequence
EVQLVESGGGLVQPGGSLRLSCVCVSSGCT

SEQ ID NO: 68 - protein, 30 aa, Artificial Sequence
  GLEW-class Nanobody FW1 sequence
EVQLVESGGGLALPGGSLTLSCVFSGSTFS

SEQ ID NO: 69 - protein, 22 aa, Artificial Sequence
  GLEW-class Nanobody FW1 sequence
VESGGGLVQPGGSLRLSCAASG

SEQ ID NO: 70 - protein, 22 aa, Artificial Sequence
  GLEW-class Nanobody FW1 sequence
EESGGGLAQPGGSLRLSCVASG

SEQ ID NO: 71 - protein, 22 aa, Artificial Sequence
  GLEW-class Nanobody FW1 sequence
VESGGGLALPGGSLTLSCVFSG

SEQ ID NO: 72 - protein, 14 aa, Artificial Sequence
  GLEW-class Nanobody FW2 sequence
WVRQAPGKVLEWVS

SEQ ID NO: 73 - protein, 14 aa, Artificial Sequence
  GLEW-class Nanobody FW2 sequence
WVRRPPGKGLEWVS

SEQ ID NO: 74 - protein, 14 aa, Artificial Sequence
  GLEW-class Nanobody FW2 sequence
WVRQAPGMGLEWVS

SEQ ID NO: 75 - protein, 14 aa, Artificial Sequence
  GLEW-class Nanobody FW2 sequence
WVRQAPGKEPEWVS

SEQ ID NO: 76 - protein, 14 aa, Artificial Sequence
  GLEW-class Nanobody FW2 sequence
WVRQAPGKDQEWVS

SEQ ID NO: 77 - protein, 14 aa, Artificial Sequence
  GLEW-class Nanobody FW2 sequence
WVRQAPGKAEEWVS

SEQ ID NO: 78 - protein, 14 aa, Artificial Sequence
  GLEW-class Nanobody FW2 sequence
WVRQAPGKGLEWVA

SEQ ID NO: 79 - protein, 14 aa, Artificial Sequence
  GLEW-class Nanobody FW2 sequence
WVRQAPGRATEWVS

SEQ ID NO: 80 - protein, 32 aa, Artificial Sequence
  GLEW-class Nanobody FW3 sequence
RFTISRDNAKNTLYLQMNSLKPEDTAVYYCVK

SEQ ID NO: 81 - protein, 32 aa, Artificial Sequence
  GLEW-class Nanobody FW3 sequence
RFTISRDNARNTLYLQMDSLIPEDTALYYCAR

SEQ ID NO: 82 - protein, 32 aa, Artificial Sequence
  GLEW-class Nanobody FW3 sequence
RFTSSRDNAKSTLYLQMNDLKPEDTALYYCAR

SEQ ID NO: 83 - protein, 32 aa, Artificial Sequence
  GLEW-class Nanobody FW3 sequence
RFIISRDNAKNTLYLQMNSLGPEDTAMYYCQR

SEQ ID NO: 84 - protein, 32 aa, Artificial Sequence
  GLEW-class Nanobody FW3 sequence
RFTASRDNAKNTLYLQMNSLKSEDTARYYCAR

SEQ ID NO: 85 - protein, 32 aa, Artificial Sequence
  GLEW-class Nanobody FW3 sequence
RFTISRDNAKNTLYLQMDDLQSEDTAMYYCGR

SEQ ID NO: 86 - protein, 11 aa, Artificial Sequence
  GLEW-class Nanobody FW4 sequence
GSQGTQVTVSS

SEQ ID NO: 87 - protein, 11 aa, Artificial Sequence
  GLEW-class Nanobody FW4 sequence
LRGGTQVTVSS

SEQ ID NO: 88 - protein, 11 aa, Artificial Sequence
  GLEW-class Nanobody FW4 sequence
RGQGTLVTVSS

SEQ ID NO: 89 - protein, 11 aa, Artificial Sequence
  GLEW-class Nanobody FW4 sequence
RSRGIQVTVSS

SEQ ID NO: 90 - protein, 11 aa, Artificial Sequence
  GLEW-class Nanobody FW4 sequence
WGKGTQVTVSS

SEQ ID NO: 91 - protein, 11 aa, Artificial Sequence
  GLEW-class Nanobody FW4 sequence
WGQGTQVTVSS

SEQ ID NO: 92 - protein, 30 aa, Artificial Sequence
  P,R,S 103-class Nanobody FW1 sequence
AVQLVESGGGLVQAGGSLRLSCAASGRTFS

SEQ ID NO: 93 - protein, 30 aa, Artificial Sequence
  P,R,S 103-class Nanobody FW1 sequence
QVQLQESGGGMVQPGGSLRLSCAASGFDFG

SEQ ID NO: 94 - protein, 30 aa, Artificial Sequence; identical to SEQ ID NO: 65
  P,R,S 103-class Nanobody FW1 sequence

SEQ ID NO: 95 - protein, 30 aa, Artificial Sequence
  P,R,S 103-class Nanobody FW1 sequence
QVQLAESGGGLVQPGGSLKLSCAASRTIVS

SEQ ID NO: 96 - protein, 30 aa, Artificial Sequence
  P,R,S 103-class Nanobody FW1 sequence
QEHLVESGGGLVDIGGSLRLSCAASERIFS

SEQ ID NO: 97 - protein, 30 aa, Artificial Sequence; identical to SEQ ID NO: 66
  P,R,S 103-class Nanobody FW1 sequence

SEQ ID NO: 98 - protein, 30 aa, Artificial Sequence; identical to SEQ ID NO: 67
  P,R,S 103-class Nanobody FW1 sequence

SEQ ID NO: 99 - protein, 30 aa, Artificial Sequence; identical to SEQ ID NO: 68
  P,R,S 103-class Nanobody FW1 sequence

SEQ ID NO: 100 - protein, 22 aa, Artificial Sequence
  P,R,S 103-class Nanobody FW1 sequence
VESGGGLVQAGGSLRLSCAASG

SEQ ID NO: 101 - protein, 22 aa, Artificial Sequence
  P,R,S 103-class Nanobody FW1 sequence
AESGGGLVQPGGSLKLSCAASR

SEQ ID NO: 102 - protein, 14 aa, Artificial Sequence
  P,R,S 103-class Nanobody FW2 sequence
WFRQAPGKEREFVA

SEQ ID NO: 103 - protein, 14 aa, Artificial Sequence
  P,R,S 103-class Nanobody FW2 sequence
WVRQAPGKVLEWVS

SEQ ID NO: 104 - protein, 14 aa, Artificial Sequence
  P,R,S 103-class Nanobody FW2 sequence
WVRRPPGKGLEWVS

SEQ ID NO: 105 - protein, 14 aa, Artificial Sequence
  P,R,S 103-class Nanobody FW2 sequence
WIRQAPGKEREGVS

SEQ ID NO: 106 - protein, 14 aa, Artificial Sequence
  P,R,S 103-class Nanobody FW2 sequence
WVRQYPGKEPEWVS

SEQ ID NO: 107 - protein, 14 aa, Artificial Sequence
  P,R,S 103-class Nanobody FW2 sequence
WFRQPPGKEHEFVA

SEQ ID NO: 108 - protein, 14 aa, Artificial Sequence
  P,R,S 103-class Nanobody FW2 sequence
WYRQAPGKRTELVA

SEQ ID NO: 109 - protein, 14 aa, Artificial Sequence
  P,R,S 103-class Nanobody FW2 sequence
WLRQAPGQGLEWVS

SEQ ID NO: 110 - protein, 14 aa, Artificial Sequence
  P,R,S 103-class Nanobody FW2 sequence
WLRQTPGKGLEWVG

SEQ ID NO: 111 - protein, 14 aa, Artificial Sequence
  P,R,S 103-class Nanobody FW2 sequence
WVRQAPGKAEEFVS

SEQ ID NO: 112 - protein, 32 aa, Artificial Sequence
  P,R,S 103-class Nanobody FW3 sequence
RFTISRDNAKNTVYLQMNSLKPEDTAVYYCAA

SEQ ID NO: 113 - protein, 32 aa, Artificial Sequence; identical to SEQ ID NO: 81
  P,R,S 103-class Nanobody FW3 sequence

SEQ ID NO: 114 - protein, 32 aa, Artificial Sequence
  P,R,S 103-class Nanobody FW3 sequence
RFTISRDNAKNEMYLQMNNLKTEDTGVYWCGA

SEQ ID NO: 115 - protein, 32 aa, Artificial Sequence
  P,R,S 103-class Nanobody FW3 sequence
RFTISSDSNRNMIYLQMNNLKPEDTAVYYCAA

SEQ ID NO: 116 - protein, 32 aa, Artificial Sequence
  P,R,S 103-class Nanobody FW3 sequence
RFTISRDNAKNMLYLHLNNLKSEDTAVYYCRR

SEQ ID NO: 117 - protein, 32 aa, Artificial Sequence
  P,R,S 103-class Nanobody FW3 sequence
RFTISRDNAKKTVYLRLNSLNPEDTAVYSCNL

SEQ ID NO: 118 - protein, 32 aa, Artificial Sequence
  P,R,S 103-class Nanobody FW3 sequence
RFKISRDNAKKTLYLQMNSLGPEDTAMYYCQR

SEQ ID NO: 119 - protein, 32 aa, Artificial Sequence
  P,R,S 103-class Nanobody FW3 sequence
RFTVSRDNGKNTAYLRMNSLKPEDTADYYCAV

SEQ ID NO: 120 - protein, 11 aa, Artificial Sequence
  P,R,S 103-class Nanobody FW4 sequence
RGQGTQVTVSS

SEQ ID NO: 121 - protein, 11 aa, Artificial Sequence
  P,R,S 103-class Nanobody FW4 sequence
LRGGTQVTVSS

SEQ ID NO: 122 - protein, 11 aa, Artificial Sequence
  P,R,S 103-class Nanobody FW4 sequence
GNKGTLVTVSS

SEQ ID NO: 123 - protein, 11 aa, Artificial Sequence
  P,R,S 103-class Nanobody FW4 sequence
SSPGTQVTVSS

SEQ ID NO: 124 - protein, 11 aa, Artificial Sequence
  P,R,S 103-class Nanobody FW4 sequence
SSQGTLVTVSS

SEQ ID NO: 125 - protein, 11 aa, Artificial Sequence
  P,R,S 103-class Nanobody FW4 sequence
RSRGIQVTVSS

SEQ ID NO: 126 - protein, 30 aa, Artificial Sequence
  Framework sequence
EVQLVESGGGLVQAGGSLRLSCAASRSIGR

SEQ ID NO: 127 - protein, 30 aa, Artificial Sequence
  Framework sequence
EVQLVESGGGLVQAGGSLRLSCVASGRSFS

SEQ ID NO: 128 - protein, 30 aa, Artificial Sequence
  Framework sequence
EVQLVESGGGLVQAGGSLRLSCAASGRTFS

SEQ ID NO: 129 - protein, 30 aa, Artificial Sequence
  Framework sequence
EVQLVESGGGLVQAGDSLRLSCAASGLTFS

SEQ ID NO: 130 - protein, 30 aa, Artificial Sequence
  Framework sequence
EVQLVESGGGLVQAGGSLRLSCAASRNILS

SEQ ID NO: 131 - protein, 30 aa, Artificial Sequence
  Framework sequence
EVQLVESGGGLVQAGGSLRLSCAASGFTLD

SEQ ID NO: 132 - protein, 30 aa, Artificial Sequence
  Framework sequence
EVQLVESGGGLVQAGASLRLSCAASGRRFI

SEQ ID NO: 133 - protein, 5 aa, Artificial Sequence
  CDR sequence
LDRMG

SEQ ID NO: 134 - protein, 5 aa, Artificial Sequence
  CDR sequence
TYIMG

SEQ ID NO: 135 - protein, 6 aa, Artificial Sequence
  CDR sequence
SIYAKG

SEQ ID NO: 136 - protein, 5 aa, Artificial Sequence
  CDR sequence
SFAMG

SEQ ID NO: 137 - protein, 5 aa, Artificial Sequence
  CDR sequence
LNTMG

SEQ ID NO: 138 - protein, 5 aa, Artificial Sequence
  CDR sequence
DYAIA

SEQ ID NO: 139 - protein, 6 aa, Artificial Sequence
  CDR sequence
SNYAMG

SEQ ID NO: 140 - protein, 14 aa, Artificial Sequence
  Framework sequence
WYRHRTGEPRELVA

SEQ ID NO: 141 - protein, 14 aa, Artificial Sequence
  Framework sequence
WFRQAPGKEREFVA

SEQ ID NO: 142 - protein, 14 aa, Artificial Sequence
  Framework sequence
WFRQAPGKEREFVA

SEQ ID NO: 143 - protein, 14 aa, Artificial Sequence
  Framework sequence
WFRQAPGKEREFVA

SEQ ID NO: 144 - protein, 14 aa, Artificial Sequence
  Framework sequence
WYRHAPGKPRELVA

SEQ ID NO: 145 - protein, 14 aa, Artificial Sequence
  Framework sequence
WFRQAPGKEREGVS

SEQ ID NO: 146 - protein, 14 aa, Artificial Sequence
  Framework sequence
WFRQAPGQERAFVA

SEQ ID NO: 147 - protein, 16 aa, Artificial Sequence
  CDR sequence
TITGGSSINYGDFVKG

SEQ ID NO: 148 - protein, 17 aa, Artificial Sequence
  CDR sequence
TISRSGITTRSADSVKG

SEQ ID NO: 149 - protein, 17 aa, Artificial Sequence
  CDR sequence
AISRSGRSTSYADSVKG

SEQ ID NO: 150 - protein, 17 aa, Artificial Sequence
  CDR sequence
AISRSGYGTSEADSVRD

SEQ ID NO: 151 - protein, 16 aa, Artificial Sequence
  CDR sequence
RISSNSKTDYADSVKG

SEQ ID NO: 152 - protein, 17 aa, Artificial Sequence
  CDR sequence
RIKISNGRTTYAGSVKG

SEQ ID NO: 153 - protein, 17 aa, Artificial Sequence
  CDR sequence
AISRSGSITYYTDSVKG

SEQ ID NO: 154 - protein, 32 aa, Artificial Sequence
  Framework sequence
RFTISIDNAKNTVYLQMNNLKPEDTAVYYCNF

SEQ ID NO: 155 - protein, 32 aa, Artificial Sequence; identical to SEQ ID NO: 112
  Framework sequence

SEQ ID NO: 156 - protein, 32 aa, Artificial Sequence; identical to SEQ ID NO: 112
  Framework sequence

SEQ ID NO: 157 - protein, 32 aa, Artificial Sequence
  Framework sequence
RFIISRDNAKNTVTLHLSRLKPEDTAVYYCAA

SEQ ID NO: 158 - protein, 32 aa, Artificial Sequence
  Framework sequence
RFTISRDNAKNTVLLQMNSLKPEDTGVYYCNL

SEQ ID NO: 159 - protein, 32 aa, Artificial Sequence
  Framework sequence
RFTISSDNAKNTVYLQMNSLNAEDTAVYYCAA

SEQ ID NO: 160 - protein, 32 aa, Artificial Sequence
  Framework sequence
RFSISRDYAKSTVYLQMDNLKPEDTAVYYCAA

SEQ ID NO: 161 - protein, 9 aa, Artificial Sequence
  CDR sequence
NKYVTSRDT

SEQ ID NO: 162 - protein, 19 aa, Artificial Sequence
  CDR sequence
GPYVEQTLGLYQTLGPWDY

SEQ ID NO: 163 - protein, 14 aa, Artificial Sequence
  CDR sequence
VGGATTVTASEWDY

SEQ ID NO: 164 - protein, 16 aa, Artificial Sequence
  CDR sequence
EHTLGRPSRSQINYLY

SEQ ID NO: 165 - protein, 9 aa, Artificial Sequence
  CDR sequence
NVWRTSSDY

SEQ ID NO: 166 - protein, 19 aa, Artificial Sequence
  CDR sequence
DRSSLLFGSNWDRKARYDY

SEQ ID NO: 167 - protein, 15 aa, Artificial Sequence
  CDR sequence
DGGAVRDLTTNLPDY

SEQ ID NO: 168 - protein, 11 aa, Artificial Sequence
  Framework sequence
WGQGTQVTVSS

SEQ ID NO: 169 - protein, 11 aa, Artificial Sequence
  Framework sequence
WGQGTQVTVSS

SEQ ID NO: 170 - protein, 11 aa, Artificial Sequence
  Framework sequence
WGLGTQVTVSS

SEQ ID NO: 171 - protein, 11 aa, Artificial Sequence
  Framework sequence
WGQGTQVTVSS

SEQ ID NO: 172 - protein, 11 aa, Artificial Sequence
  Framework sequence
WGQGTQVTVSS

SEQ ID NO: 173 - protein, 11 aa, Artificial Sequence
  Framework sequence
WGQGTQVTVSS

SEQ ID NO: 174 - protein, 11 aa, Artificial Sequence
  Framework sequence
WGRGTQVTVSS

SEQ ID NO: 175 - protein, 183 aa, Homo sapiens
MERVQPLEENVGNAARPRFERNKLLLVASVIQGLGLLLCFTYICLHFSALQVSHRYPRIQSIKVQFTEYKKEKGFILTSQKEDEIMKVQNNSVIINCDGFYLISLKGYFSQEVNISLHYQKDEEPLFQLKKVRSVNSLMVASLTYKDKVYLNVTTDNTSLDDFHVNGGELILIHQNPGEFCVL

SEQ ID NO: 176 - protein, 183 aa, Macaca fascicularis
MERVQPLEENVGNAARPRFERNKLLLVASVIQGLGLLLCFTYICLHFSALQVSHQYPRIQSIKVQFTEYKKEEGFILTSQKEDEIMKVQNNSVIINCDGFYLISLKGYFSQEVNISLHYQKDEEPLFQLKKVRSVNSLMVASLTYKDKVYLNVTTDNTSLDDFHVNGGELILIHQNPGEFCVL

SEQ ID NO: 177 - protein, 450 aa, Artificial Sequence
  Antibody heavy chain
EVQLLESGGGLVQPGGSLRLSCAASGFTFNSYAMSWVRQAPGKGLEWVSIISGSGGFTYYADSVKGRFTISRDNSRTTLYLQMNSLRAEDTAVYYCAKDRLVAPGTFDYWGQGALVTVSSASTKGPSVFPLAPSSKSTSGGTAALGCLVKDYFPEPVTVSWNSGALTSGVHTFPAVLQSSGLYSLSSVVTVPSSSLGTQTYICNVNHKPSNTKVDKKVEPKSCDKTHTCPPCPAPELLGGPSVFLFPPKPKDTLMISRTPEVTCVVVDVSHEDPEVKFNWYVDGVEVHNAKTKPREEQYNSTYRVVSVLTVLHQDWLNGKEYKCKVSNKALPAPIEKTISKAKGQPREPQVYTLPPSRDELTKNQVSLTCLVKGFYPSDIAVEWESNGQPENNYKTTPPVLDSDGSFFLYSKLTVDKSRWQQGNVFSCSVMHEALHNHYTQKSLSLSPGK

SEQ ID NO: 178 - protein, 214 aa, Artificial Sequence
  Antibody light chain
DIQMTQSPSSLSASVGDRVTITCRASQGISSWLAWYQQKPEKAPKSLIYAASSLQSGVPSRFSGSGSGTDFTLTISSLQPEDFATYYCQQYNSYPYTFGQGTKLEIKRTVAAPSVFIFPPSDEQLKSGTASVVCLLNNFYPREAKVQWKVDNALQSGNSQESVTEQDSKDSTYSLSSTLTLSKADYEKHKVYACEVTHQGLSSPVTKSFNRGEC

SEQ ID NO: 179 - protein, 117 aa, Artificial Sequence
  Nanobody sequence
EVQLVESGGGLVQAGGSLRLSCAASRSIGRLDRMGWYRHRTGEPRELVATITGGSSINYGDFVKGRFTISIDNAKNTVYLQMNNLKPEDTAVYYCNFNKYVTSRDTWGQGTQVTVSS

SEQ ID NO: 180 - protein, 128 aa, Artificial Sequence
  Nanobody sequence
EVQLVESGGGLVQAGGSLRLSCVASGRSFSTYIMGWFRQAPGKEREFVATISRSGITTRSADSVKGRFTISRDNAKNTVYLQMNSLKPEDTAVYYCAAGPYVEQTLGLYQTLGPWDYWGQGTQVTVSS

SEQ ID NO: 181 - protein, 124 aa, Artificial Sequence
  Nanobody sequence
EVQLVESGGGLVQAGGSLRLSCAASGRTFSSIYAKGWFRQAPGKEREFVAAISRSGRSTSYADSVKGRFTISRDNAKNTVYLQMNSLKPEDTAVYYCAAVGGATTVTASEWDYWGLGTQVTVSS

SEQ ID NO: 182 - protein, 125 aa, Artificial Sequence
  Nanobody sequence
EVQLVESGGGLVQAGDSLRLSCAASGLTFSSFAMGWFRQAPGKEREFVAAISRSGYGTSEADSVRDRFIISRDNAKNTVTLHLSRLKPEDTAVYYCAAEHTLGRPSRSQINYLYWGQGTQVTVSS

SEQ ID NO: 183 - protein, 117 aa, Artificial Sequence
  Nanobody sequence
EVQLVESGGGLVQAGGSLRLSCAASRNILSLNTMGWYRHAPGKPRELVARISSNSKTDYADSVKGRFTISRDNAKNTVLLQMNSLKPEDTGVYYCNLNVWRTSSDYWGQGTQVTVSS

SEQ ID NO: 184 - protein, 128 aa, Artificial Sequence
  Nanobody sequence
EVQLVESGGGLVQAGGSLRLSCAASGFTLDDYAIAWFRQAPGKEREGVSRIKISNGRTTYAGSVKGRFTISSDNAKNTVYLQMNSLNAEDTAVYYCAADRSSLLFGSNWDRKARYDYWGQGTQVTVSS

SEQ ID NO: 185 - protein, 125 aa, Artificial Sequence
  Nanobody sequence
EVQLVESGGGLVQAGASLRLSCAASGRRFISNYAMGWFRQAPGQERAFVAAISRSGSITYYTDSVKGRFSISRDYAKSTVYLQMDNLKPEDTAVYYCAADGGAVRDLTTNLPDYWGRGTQVTVSS

SEQ ID NO: 186 - protein, 381 aa, Artificial Sequence
  Nanobody sequence
EVQLVESGGGLVQAGGSLRLSCAASGRTFSSIYAKGWFRQAPGKEREFVAAISRSGRSTSYADSVKGRFTISRDNAKNTVYLQMNSLKPEDTAVYYCAAVGGATTVTASEWDYWGLGTQVTVSSGGGGSGGGSEVQLVESGGGLVQPGNSLRLSCAASGFTFSSFGMSWVRQAPGKGLEWVSSISGSGSDTLYADSVKGRFTISRDNAKTTLYLQMNSLRPEDTAVYYCTIGGSLSRSSQGTLVTVSSGGGGSGGGSEVQLVESGGGLVQAGGSLRLSCAASGRTFSSIYAKGWFRQAPGKEREFVAAISRSGRSTSYADSVKGRFTISRDNAKNTVYLQMNSLKPEDTAVYYCAAVGGATTVTASEWDYWGLGTQVTVSS

SEQ ID NO: 187 - protein, 367 aa, Artificial Sequence
  Nanobody sequence
EVQLVESGGGLVQAGGSLRLSCAASRNILSLNTMGWYRHAPGKPRELVARISSNSKTDYADSVKGRFTISRDNAKNTVLLQMNSLKPEDTGVYYCNLNVWRTSSDYWGQGTQVTVSSGGGGSGGGSEVQLVESGGGLVQPGNSLRLSCAASGFTFSSFGMSWVRQAPGKGLEWVSSISGSGSDTLYADSVKGRFTISRDNAKTTLYLQMNSLRPEDTAVYYCTIGGSLSRSSQGTLVTVSSGGGGSGGGSEVQLVESGGGLVQAGGSLRLSCAASRNILSLNTMGWYRHAPGKPRELVARISSNSKTDYADSVKGRFTISRDNAKNTVLLQMNSLKPEDTGVYYCNLNVWRTSSDYWGQGTQVTVSS

SEQ ID NO: 188 - protein, 383 aa, Artificial Sequence
  Nanobody sequence
EVQLVESGGGLVQAGASLRLSCAASGRRFISNYAMGWFRQAPGQERAFVAAISRSGSITYYTDSVKGRFSISRDYAKSTVYLQMDNLKPEDTAVYYCAADGGAVRDLTTNLPDYWGRGTQVTVSSGGGGSGGGSEVQLVESGGGLVQPGNSLRLSCAASGFTFSSFGMSWVRQAPGKGLEWVSSISGSGSDTLYADSVKGRFTISRDNAKTTLYLQMNSLRPEDTAVYYCTIGGSLSRSSQGTLVTVSSGGGGSGGGSEVQLVESGGGLVQAGASLRLSCAASGRRFISNYAMGWFRQAPGQERAFVAAISRSGSITYYTDSVKGRFSISRDYAKSTVYLQMDNLKPEDTAVYYCAADGGAVRDLTTNLPDYWGRGTQVTVSS

SEQ ID NO: 189 - protein, 383 aa, Artificial Sequence
  Nanobody sequence
EVQLVESGGGLVQAGDSLRLSCAASGLTFSSFAMGWFRQAPGKEREFVAAISRSGYGTSEADSVRDRFIISRDNAKNTVTLHLSRLKPEDTAVYYCAAEHTLGRPSRSQINYLYWGQGTQVTVSSGGGGSGGGSEVQLVESGGGLVQPGNSLRLSCAASGFTFSSFGMSWVRQAPGKGLEWVSSISGSGSDTLYADSVKGRFTISRDNAKTTLYLQMNSLRPEDTAVYYCTIGGSLSRSSQGTLVTVSSGGGGSGGGSEVQLVESGGGLVQAGDSLRLSCAASGLTFSSFAMGWFRQAPGKEREFVAAISRSGYGTSEADSVRDRFIISRDNAKNTVTLHLSRLKPEDTAVYYCAAEHTLGRPSRSQINYLYWGQGTQVTVSS

SEQ ID NO: 190 - protein, 367 aa, Artificial Sequence
  Nanobody sequence
EVQLVESGGGLVQAGGSLRLSCAASRSIGRLDRMGWYRHRTGEPRELVATITGGSSINYGDFVKGRFTISIDNAKNTVYLQMNNLKPEDTAVYYCNFNKYVTSRDTWGQGTQVTVSSGGGGSGGGSEVQLVESGGGLVQPGNSLRLSCAASGFTFSSFGMSWVRQAPGKGLEWVSSISGSGSDTLYADSVKGRFTISRDNAKTTLYLQMNSLRPEDTAVYYCTIGGSLSRSSQGTLVTVSSGGGGSGGGSEVQLVESGGGLVQAGGSLRLSCAASRSIGRLDRMGWYRHRTGEPRELVATITGGSSINYGDFVKGRFTISIDNAKNTVYLQMNNLKPEDTAVYYCNFNKYVTSRDTWGQGTQVTVSS

SEQ ID NO: 191 - protein, 389 aa, Artificial Sequence
  Nanobody sequence
EVQLVESGGGLVQAGGSLRLSCAASGFTLDDYAIAWFRQAPGKEREGVSRIKISNGRTTYAGSVKGRFTISSDNAKNTVYLQMNSLNAEDTAVYYCAADRSSLLFGSNWDRKARYDYWGQGTQVTVSSGGGGSGGGSEVQLVESGGGLVQPGNSLRLSCAASGFTFSSFGMSWVRQAPGKGLEWVSSISGSGSDTLYADSVKGRFTISRDNAKTTLYLQMNSLRPEDTAVYYCTIGGSLSRSSQGTLVTVSSGGGGSGGGSEVQLVESGGGLVQAGGSLRLSCAASGFTLDDYAIAWFRQAPGKEREGVSRIKISNGRTTYAGSVKGRFTISSDNAKNTVYLQMNSLNAEDTAVYYCAADRSSLLFGSNWDRKARYDYWGQGTQVTVSS

SEQ ID NO: 192 - protein, 389 aa, Artificial Sequence; identical to SEQ ID NO: 191
  Nanobody sequence

SEQ ID NO: 193 - protein, 407 aa, Artificial Sequence
  Nanobody sequence
EVQLVESGGGLVQAGGSLRLSCAASGRTFSSIYAKGWFRQAPGKEREFVAAISRSGRSTSYADSVKGRFTISRDNAKNTVYLQMNSLKPEDTAVYYCAAVGGATTVTASEWDYWGLGTLVTVSSGGGGSGGGGSGGGGSGGGGSGGGGSGGGGSGGGGSEVQLVESGGGLVQAGGSLRLSCAASGRTFSSIYAKGWFRQAPGKEREFVAAISRSGRSTSYADSVKGRFTISRDNAKNTVYLQMNSLKPEDTAVYYCAAVGGATTVTASEWDYWGLGTLVTVSSGGGGSGGGSEVQLVESGGGLVQPGNSLRLSCAASGFTFSSFGMSWVRQAPGKGLEWVSSISGSGSDTLYADSVKGRFTISRDNAKTTLYLQMNSLRPEDTAVYYCTIGGSLSRSSQGTLVTVSS

SEQ ID NO: 194 - protein, 433 aa, Artificial Sequence
  Nanobody sequence
EVQLVESGGGLVQAGGSLRLSCAASGRTFSSIYAKGWFRQAPGKEREFVAAISRSGRSTSYADSVKGRFTISRDNAKNTVYLQMNSLKPEDTAVYYCAAVGGATTVTASEWDYWGLGTLVTVSSGGGGSGGGGSGGGGSGGGGSGGGGSGGGGSGGGGSEVQLVESGGGLVQAGGSLRLSCAASGRTFSSIYAKGWFRQAPGKEREFVAAISRSGRSTSYADSVKGRFTISRDNAKNTVYLQMNSLKPEDTAVYYCAAVGGATTVTASEWDYWGLGTLVTVSSGGGGSGGGGSGGGGSGGGGSGGGGSGGGGSGGGGSEVQLVESGGGLVQPGNSLRLSCAASGFTFSSFGMSWVRQAPGKGLEWVSSISGSGSDTLYADSVKGRFTISRDNAKTTLYLQMNSLRPEDTAVYYCTIGGSLSRSSQGTLVTVSS

SEQ ID NO: 195 - protein, 409 aa, Artificial Sequence
  Nanobody sequence
EVQLVESGGGLVQAGDSLRLSCAASGLTFSSFAMGWFRQAPGKEREFVAAISRSGYGTSEADSVRDRFIISRDNAKNTVTLHLSRLKPEDTAVYYCAAEHTLGRPSRSQINYLYWGQGTLVTVSSGGGGSGGGGSGGGGSGGGGSGGGGSGGGGSGGGGSEVQLVESGGGLVQAGDSLRLSCAASGLTFSSFAMGWFRQAPGKEREFVAAISRSGYGTSEADSVRDRFIISRDNAKNTVTLHLSRLKPEDTAVYYCAAEHTLGRPSRSQINYLYWGQGTLVTVSSGGGGSGGGSEVQLVESGGGLVQPGNSLRLSCAASGFTFSSFGMSWVRQAPGKGLEWVSSISGSGSDTLYADSVKGRFTISRDNAKTTLYLQMNSLRPEDTAVYYCTIGGSLSRSSQGTLVTVSS

SEQ ID NO: 196 - protein, 435 aa, Artificial Sequence
  Nanobody sequence
EVQLVESGGGLVQAGDSLRLSCAASGLTFSSFAMGWFRQAPGKEREFVAAISRSGYGTSEADSVRDRFIISRDNAKNTVTLHLSRLKPEDTAVYYCAAEHTLGRPSRSQINYLYWGQGTLVTVSSGGGGSGGGGSGGGGSGGGGSGGGGSGGGGSGGGGSEVQLVESGGGLVQAGDSLRLSCAASGLTFSSFAMGWFRQAPGKEREFVAAISRSGYGTSEADSVRDRFIISRDNAKNTVTLHLSRLKPEDTAVYYCAAEHTLGRPSRSQINYLYWGQGTLVTVSSGGGGSGGGGSGGGGSGGGGSGGGGSGGGGSGGGGSEVQLVESGGGLVQPGNSLRLSCAASGFTFSSFGMSWVRQAPGKGLEWVSSISGSGSDTLYADSVKGRFTISRDNAKTTLYLQMNSLRPEDTAVYYCTIGGSLSRSSQGTLVTVSS

SEQ ID NO: 197 - protein, 393 aa, Artificial Sequence
  Nanobody sequence
EVQLVESGGGLVQAGGSLRLSCAASRSIGRLDRMGWYRHRTGEPRELVATITGGSSINYGDFVKGRFTISIDNAKNTVYLQMNNLKPEDTAVYYCNFNKYVTSRDTWGQGTLVTVSSGGGGSGGGGSGGGGSGGGGSGGGGSGGGGSGGGGSEVQLVESGGGLVQAGGSLRLSCAASRSIGRLDRMGWYRHRTGEPRELVATITGGSSINYGDFVKGRFTISIDNAKNTVYLQMNNLKPEDTAVYYCNFNKYVTSRDTWGQGTLVTVSSGGGGSGGGSEVQLVESGGGLVQPGNSLRLSCAASGFTFSSFGMSWVRQAPGKGLEWVSSISGSGSDTLYADSVKGRFTISRDNAKTTLYLQMNSLRPEDTAVYYCTIGGSLSRSSQGTLVTVSS

SEQ ID NO: 198 - protein, 419 aa, Artificial Sequence
  Nanobody sequence
EVQLVESGGGLVQAGGSLRLSCAASRSIGRLDRMGWYRHRTGEPRELVATITGGSSINYGDFVKGRFTISIDNAKNTVYLQMNNLKPEDTAVYYCNFNKYVTSRDTWGQGTLVTVSSGGGGSGGGGSGGGGSGGGGSGGGGSGGGGSGGGGSEVQLVESGGGLVQAGGSLRLSCAASRSIGRLDRMGWYRHRTGEPRELVATITGGSSINYGDFVKGRFTISIDNAKNTVYLQMNNLKPEDTAVYYCNFNKYVTSRDTWGQGTLVTVSSGGGGSGGGGSGGGGSGGGGSGGGGSGGGGSGGGGSEVQLVESGGGLVQPGNSLRLSCAASGFTFSSFGMSWVRQAPGKGLEWVSSISGSGSDTLYADSVKGRFTISRDNAKTTLYLQMNSLRPEDTAVYYCTIGGSLSRSSQGTLVTVSS

SEQ ID NO: 199 - protein, 128 aa, Artificial Sequence
  Nanobody sequence
EVQLVESGGGLVQPGGSLRLSCAASGRSFSTYIMGWFRQAPGKEREFVATISRSGITTRSADSVKGRFTISRDNSKNTVYLQMNSLRPEDTAVYYCAAGPYVEQTLGLYQTLGPWDYWGQGTLVTVSS

SEQ ID NO: 200 - protein, 124 aa, Artificial Sequence
  Nanobody sequence
EVQLVESGGGLVQPGGSLRLSCAASGRTFSSIYAKGWFRQAPGKEREFVAAISRSGRSTSYADSVKGRFTISRDNAKNTVYLQMNSLRPEDTAVYYCAAVGGATTVTASEWDYWGLGTLVTVSS

SEQ ID NO: 201 - protein, 124 aa, Artificial Sequence
  Nanobody sequence
EVQLVESGGGLVQPGGSLRLSCAASGRTFSSIYAKGWFRQAPGKEREFVAAISRSGRSTSYADSVKGRFTISRDNSKNTVYLQMNSLRPEDTAVYYCAAVGGATTVTASEWDYWGLGTLVTVSS

SEQ ID NO: 202 - protein, 124 aa, Artificial Sequence
  Nanobody sequence
EVQLVESGGGLVQPGGSLRLSCAASGRTFSSIYAKGWFRQAPGKEREFVAAISRSGRSTSYADSVKGRFTISRDNAKNTVYLQMNSLRPEDTAVYYCAAVGGATTVTASEWDYWGQGTLVTVSS

SEQ ID NO: 203 - protein, 124 aa, Artificial Sequence
  Nanobody sequence
EVQLVESGGGLVQPGGSLRLSCAASGRTFSSIYAKGWFRQAPGKEREFVAAISRSGRSTSYADSVKGRFTISRDNSKNTVYLQMNSLRPEDTAVYYCAAVGGATTVTASEWDYWGQGTLVTVSS

SEQ ID NO: 204 - protein, 124 aa, Artificial Sequence
  Nanobody sequence
DVQLVESGGGLVQPGGSLRLSCAASGRTFSSIYAKGWFRQAPGKEREFVAAISRSGRSTSYADSVKGRFTISRDNAKNTVYLQMNSLRPEDTAVYYCAAVGGATTVTASEWDYWGLGTLVTVSS

SEQ ID NO: 205 - protein, 124 aa, Artificial Sequence
  Nanobody sequence
DVQLVESGGGLVQPGGSLRLSCAASGRTFSSIYAKGWFRQAPGKEREFVAAISRSGRSTSYADSVKGRFTISRDNSKNTVYLQMNSLRPEDTAVYYCAAVGGATTVTASEWDYWGQGTLVTVSS

SEQ ID NO: 206 - protein, 117 aa, Artificial Sequence
  Nanobody sequence
DVQLVESGGGLVQAGGSLRLSCAASRSIGRLDRMGWYRHRTGEPRELVATITGGSSINYGDFVKGRFTISIDNAKNTVYLQMNNLKPEDTAVYYCNFNKYVTSRDTWGQGTQVTVSS

SEQ ID NO: 207 - protein, 117 aa, Artificial Sequence
  Nanobody sequence
DVQLVESGGGLVQPGGSLRLSCAASRSIGRLDRMGWYRHRTGEPRELVATITGGSSINYGDFVKGRFTISRDNSKNTVYLQMNSLRPEDTAVYYCNFNKYVTSRDTWGQGTLVTVSS

SEQ ID NO: 208 - protein, 117 aa, Artificial Sequence
  Nanobody sequence
DVQLVESGGGLVQPGGSLRLSCAASRSIGRLDRMGWYRHATGEPRELVATITGGSSINYGDFVKGRFTISRDNSKNTVYLQMNSLRPEDTAVYYCNFNKYVTSRDTWGQGTLVTVSS

SEQ ID NO: 209 - protein, 117 aa, Artificial Sequence
  Nanobody sequence
DVQLVESGGGLVQPGGSLRLSCAASRSIGRLDRMGWYRHRPGEPRELVATITGGSSINYGDFVKGRFTISRDNSKNTVYLQMNSLRPEDTAVYYCNFNKYVTSRDTWGQGTLVTVSS

SEQ ID NO: 210 - protein, 117 aa, Artificial Sequence
  Nanobody sequence
DVQLVESGGGLVQPGGSLRLSCAASRSIGRLDRMGWYRHRTGKPRELVATITGGSSINYGDFVKGRFTISRDNSKNTVYLQMNSLRPEDTAVYYCNFNKYVTSRDTWGQGTLVTVSS

SEQ ID NO: 211 - protein, 117 aa, Artificial Sequence
  Nanobody sequence
DVQLVESGGGLVQPGGSLRLSCAASRSIGRLDRMGWYRHAPGEPRELVATITGGSSINYGDFVKGRFTISRDNSKNTVYLQMNSLRPEDTAVYYCNFNKYVTSRDTWGQGTLVTVSS

SEQ ID NO: 212 - protein, 117 aa, Artificial Sequence
  Nanobody sequence
DVQLVESGGGLVQPGGSLRLSCAASRSIGRLDRMGWYRHATGKPRELVATITGGSSINYGDFVKGRFTISRDNSKNTVYLQMNSLRPEDTAVYYCNFNKYVTSRDTWGQGTLVTVSS

SEQ ID NO: 213 - protein, 117 aa, Artificial Sequence
  Nanobody sequence
DVQLVESGGGLVQPGGSLRLSCAASRSIGRLDRMGWYRHRPGKPRELVATITGGSSINYGDFVKGRFTISRDNSKNTVYLQMNSLRPEDTAVYYCNFNKYVTSRDTWGQGTLVTVSS

SEQ ID NO: 214 - protein, 117 aa, Artificial Sequence
  Nanobody sequence
DVQLVESGGGLVQPGGSLRLSCAASRSIGRLDRMGWYRHAPGKPRELVATITGGSSINYGDFVKGRFTISRDNSKNTVYLQMNSLRPEDTAVYYCNFNKYVTSRDTWGQGTLVTVSS

SEQ ID NO: 215 - protein, 117 aa, Artificial Sequence
  Nanobody sequence
DVQLVESGGGLVQPGGSLRLSCAASRSIGRLDRMGWYRHRTGEPRELVATITGGSSINYADFVKGRFTISRDNSKNTVYLQMNSLRPEDTAVYYCNFNKYVTSRDTWGQGTLVTVSS

SEQ ID NO: 216 - protein, 117 aa, Artificial Sequence
  Nanobody sequence
DVQLVESGGGLVQPGGSLRLSCAASRSIGRLDRMGWYRHRTGEPRELVATITGGSSINYGDSVKGRFTISRDNSKNTVYLQMNSLRPEDTAVYYCNFNKYVTSRDTWGQGTLVTVSS

SEQ ID NO: 217 - protein, 117 aa, Artificial Sequence
  Nanobody sequence
DVQLVESGGGLVQPGGSLRLSCAASRSIGRLDRMGWYRHRTGEPRELVATITGGSSINYADSVKGRFTISRDNSKNTVYLQMNSLRPEDTAVYYCNFNKYVTSRDTWGQGTLVTVSS

SEQ ID NO: 218 - protein, 117 aa, Artificial Sequence
  Nanobody sequence
DVQLVESGGGLVQPGGSLRLSCAASRSIGRLDRMGWYRHRTGEPRELVATITGGSSINYGDFVKGRFTISIDNSKNTVYLQMNSLRPEDTAVYYCNFNKYVTSRDTWGQGTLVTVSS

SEQ ID NO: 219 - protein, 117 aa, Artificial Sequence
  Nanobody sequence
DVQLVESGGGLVQPGGSLRLSCAASRSIGRLDRMGWYRHRTGEPRELVATITGGSSINYGDFVKGRFTISRDNAKNTVYLQMNSLRPEDTAVYYCNFNKYVTSRDTWGQGTLVTVSS

SEQ ID NO: 220 - protein, 117 aa, Artificial Sequence
  Nanobody sequence
DVQLVESGGGLVQPGGSLRLSCAASRSIGRLDRMGWYRHRTGEPRELVATITGGSSINYGDFVKGRFTISRDNSKNTVYLQMNNLRPEDTAVYYCNFNKYVTSRDTWGQGTLVTVSS

SEQ ID NO: 221 - protein, 117 aa, Artificial Sequence
  Nanobody sequence
DVQLVESGGGLVQPGGSLRLSCAASRSIGRLDRMGWYRHRPGKPRELVATITGGSSINYADSVKGRFTISRDNSKNTVYLQMNSLRPEDTAVYYCNFNKYVTSRDTWGQGTLVTVSS

SEQ ID NO: 222 - protein, 117 aa, Artificial Sequence
  Nanobody sequence
DVQLVESGGGLVQPGGSLRLSCAASRSIGRLDRMGWYRHRPGKPRELVATITGGSSINYADSVKGRFTISIDNSKNTVYLQMNSLRPEDTAVYYCNFNKYVTSRDTWGQGTLVTVSS

SEQ ID NO: 223 - protein, 117 aa, Artificial Sequence
  Nanobody sequence
DVQLVESGGGLVQPGGSLRLSCAASRSIGRLDRMGWYRHRPGKPRELVATITGGSSINYADSVKGRFTISRDNSKNTVYLQMNNLRPEDTAVYYCNFNKYVTSRDTWGQGTLVTVSS

SEQ ID NO: 224 - protein, 117 aa, Artificial Sequence
  Nanobody sequence
DVQLVESGGGLVQPGGSLRLSCAASRSIGRLDRMGWYRHRPGKPRELVATITGGSSINYADSVKGRFTISIDNSKNTVYLQMNNLRPEDTAVYYCNFNKYVTSRDTWGQGTLVTVSS

SEQ ID NO: 225 - protein, 117 aa, Artificial Sequence
  Nanobody sequence
EVQLVESGGGLVQPGGSLRLSCAASRSIGRLDRMGWYRHRPGEPRELVATITGGSSINYGDSVKGRFTISIDNSKNTVYLQMNSLRPEDTAVYYCNFNKYVTSRDTWGQGTLVTVSS

SEQ ID NO: 226 - protein, 117 aa, Artificial Sequence
  Nanobody sequence
EVQLVESGGGLVQPGGSLRLSCAASRSIGRLDRMGWYRHRPGKPRELVATITGGSSINYGDSVKGRFTISIDNSKNTVYLQMNSLRPEDTAVYYCNFNKYVTSRDTWGQGTLVTVSS

SEQ ID NO: 227 - protein, 441 aa, Artificial Sequence
  Nanobody sequence
EVQLVESGGGLVQPGGSLRLSCAASGRSFSTYIMGWFRQAPGKEREFVATISRSGITTRSADSVKGRFTISRDNSKNTVYLQMNSLRPEDTAVYYCAAGPYVEQTLGLYQTLGPWDYWGQGTLVTVSSGGGGSGGGGSGGGGSGGGGSGGGGSGGGGSGGGGSEVQLVESGGGLVQPGGSLRLSCAASGRSFSTYIMGWFRQAPGKEREFVATISRSGITTRSADSVKGRFTISRDNSKNTVYLQMNSLRPEDTAVYYCAAGPYVEQTLGLYQTLGPWDYWGQGTLVTVSSGGGGSGGGGSGGGGSGGGGSGGGGSGGGGSGGGGSEVQLVESGGGLVQPGNSLRLSCAASGFTFSSFGMSWVRQAPGKGLEWVSSISGSGSDTLYADSVKGRFTISRDNAKTTLYLQMNSLRPEDTAVYYCTIGGSLSRSSQGTLVTVSS

SEQ ID NO: 228 - protein, 441 aa, Artificial Sequence
  Nanobody sequence
EVQLVESGGGLVQPGGSLRLSCAASGRSFSTYIMGWFRQAPGKEREFVATISRSGITTRSADSVKGRFTISRDNSKNTVYLQMNSLRPEDTAVYYCAAGPYVEQTLGLYQTLGPWDYWGQGTLVTVSSGGGGSGGGGSGGGGSGGGGSGGGGSGGGGSGGGGSEVQLVESGGGLVQPGNSLRLSCAASGFTFSSFGMSWVRQAPGKGLEWVSSISGSGSDTLYADSVKGRFTISRDNAKTTLYLQMNSLRPEDTAVYYCTIGGSLSRSSQGTLVTVSSGGGGSGGGGSGGGGSGGGGSGGGGSGGGGSGGGGSEVQLVESGGGLVQPGGSLRLSCAASGRSFSTYIMGWFRQAPGKEREFVATISRSGITTRSADSVKGRFTISRDNSKNTVYLQMNSLRPEDTAVYYCAAGPYVEQTLGLYQTLGPWDYWGQGTLVTVSS

SEQ ID NO: 229 - protein, 433 aa, Artificial Sequence
  Nanobody sequence
DVQLVESGGGLVQPGGSLRLSCAASGRTFSSIYAKGWFRQAPGKEREFVAAISRSGRSTSYADSVKGRFTISRDNSKNTVYLQMNSLRPEDTAVYYCAAVGGATTVTASEWDYWGQGTLVTVSSGGGGSGGGGSGGGGSGGGGSGGGGSGGGGSGGGGSEVQLVESGGGLVQPGGSLRLSCAASGRTFSSIYAKGWFRQAPGKEREFVAAISRSGRSTSYADSVKGRFTISRDNSKNTVYLQMNSLRPEDTAVYYCAAVGGATTVTASEWDYWGQGTLVTVSSGGGGSGGGGSGGGGSGGGGSGGGGSGGGGSGGGGSEVQLVESGGGLVQPGNSLRLSCAASGFTFSSFGMSWVRQAPGKGLEWVSSISGSGSDTLYADSVKGRFTISRDNAKTTLYLQMNSLRPEDTAVYYCTIGGSLSRSSQGTLVTVSS

SEQ ID NO: 230 - protein, 433 aa, Artificial Sequence
  Nanobody sequence
DVQLVESGGGLVQPGGSLRLSCAASGRTFSSIYAKGWFRQAPGKEREFVAAISRSGRSTSYADSVKGRFTISRDNSKNTVYLQMNSLRPEDTAVYYCAAVGGATTVTASEWDYWGQGTLVTVSSGGGGSGGGGSGGGGSGGGGSGGGGSGGGGSGGGGSEVQLVESGGGLVQPGNSLRLSCAASGFTFSSFGMSWVRQAPGKGLEWVSSISGSGSDTLYADSVKGRFTISRDNAKTTLYLQMNSLRPEDTAVYYCTIGGSLSRSSQGTLVTVSSGGGGSGGGGSGGGGSGGGGSGGGGSGGGGSGGGGSEVQLVESGGGLVQPGGSLRLSCAASGRTFSSIYAKGWFRQAPGKEREFVAAISRSGRSTSYADSVKGRFTISRDNSKNTVYLQMNSLRPEDTAVYYCAAVGGATTVTASEWDYWGQGTLVTVSS

SEQ ID NO: 231 - protein, 367 aa, Artificial Sequence
  Nanobody sequence
DVQLVESGGGLVQPGGSLRLSCAASRSIGRLDRMGWYRHRPGEPRELVATITGGSSINYGDSVKGRFTISIDNSKNTVYLQMNSLRPEDTAVYYCNFNKYVTSRDTWGQGTLVTVSSGGGGSGGGSEVQLVESGGGLVQPGNSLRLSCAASGFTFSSFGMSWVRQAPGKGLEWVSSISGSGSDTLYADSVKGRFTISRDNAKTTLYLQMNSLRPEDTAVYYCTIGGSLSRSSQGTLVTVSSGGGGSGGGSEVQLVESGGGLVQPGGSLRLSCAASRSIGRLDRMGWYRHRPGEPRELVATITGGSSINYGDSVKGRFTISIDNSKNTVYLQMNSLRPEDTAVYYCNFNKYVTSRDTWGQGTLVTVSS

SEQ ID NO: 232 - protein, 367 aa, Artificial Sequence
  Nanobody sequence
DVQLVESGGGLVQPGGSLRLSCAASRSIGRLDRMGWYRHRPGKPRELVATITGGSSINYGDSVKGRFTISIDNSKNTVYLQMNSLRPEDTAVYYCNFNKYVTSRDTWGQGTLVTVSSGGGGSGGGSEVQLVESGGGLVQPGNSLRLSCAASGFTFSSFGMSWVRQAPGKGLEWVSSISGSGSDTLYADSVKGRFTISRDNAKTTLYLQMNSLRPEDTAVYYCTIGGSLSRSSQGTLVTVSSGGGGSGGGSEVQLVESGGGLVQPGGSLRLSCAASRSIGRLDRMGWYRHRPGKPRELVATITGGSSINYGDSVKGRFTISIDNSKNTVYLQMNSLRPEDTAVYYCNFNKYVTSRDTWGQGTLVTVSS

SEQ ID NO: 233 - protein, 441 aa, Artificial Sequence
  Nanobody sequence
DVQLVESGGGLVQPGGSLRLSCAASGRSFSTYIMGWFRQAPGKEREFVATISRSGITTRSADSVKGRFTISRDNSKNTVYLQMNSLRPEDTAVYYCAAGPYVEQTLGLYQTLGPWDYWGQGTLVTVSSGGGGSGGGGSGGGGSGGGGSGGGGSGGGGSGGGGSEVQLVESGGGLVQPGNSLRLSCAASGFTFSSFGMSWVRQAPGKGLEWVSSISGSGSDTLYADSVKGRFTISRDNAKTTLYLQMNSLRPEDTAVYYCTIGGSLSRSSQGTLVTVSSGGGGSGGGGSGGGGSGGGGSGGGGSGGGGSGGGGSEVQLVESGGGLVQPGGSLRLSCAASGRSFSTYIMGWFRQAPGKEREFVATISRSGITTRSADSVKGRFTISRDNSKNTVYLQMNSLRPEDTAVYYCAAGPYVEQTLGLYQTLGPWDYWGQGTLVTVSS

SEQ ID NO: 234 - protein, 389 aa, Artificial Sequence
  Nanobody sequence
DVQLVESGGGLVQPGGSLRLSCAASGRSFSTYIMGWFRQAPGKEREFVATISRSGITTRSADSVKGRFTISRDNSKNTVYLQMNSLRPEDTAVYYCAAGPYVEQTLGLYQTLGPWDYWGQGTLVTVSSGGGGSGGGSEVQLVESGGGLVQPGNSLRLSCAASGFTFSSFGMSWVRQAPGKGLEWVSSISGSGSDTLYADSVKGRFTISRDNAKTTLYLQMNSLRPEDTAVYYCTIGGSLSRSSQGTLVTVSSGGGGSGGGSEVQLVESGGGLVQPGGSLRLSCAASGRSFSTYIMGWFRQAPGKEREFVATISRSGITTRSADSVKGRFTISRDNSKNTVYLQMNSLRPEDTAVYYCAAGPYVEQTLGLYQTLGPWDYWGQGTLVTVSS